European Patent Specification EP 3 805 385 B1, published October 30, 2024. Title: LENTIVIRAL VECTOR AND METHOD FOR DELIVERING EXOGENOUS RNA BY THE LENTIVIRAL VECTOR. Applicant: SHANGHAI BDGENE TECHNOLOGY CO., LTD. The sequence listing filed with the application follows.

SEQUENCE LISTING (3 sequences)

SEQ ID NO: 1 - DNA, 4337 bp, Artificial Sequence
  The sequence is synthetized.
  misc_feature: codon sequence of GagPol long-chain protein
gccagggccagcgtgctgagcggcggcgagctggacaggtgggagaagatcaggctgaggcccggcggcaagaagaagtataagctgaagcacatcgtgtgggccagcagggagctggagaggttcgccgtgaaccccggcctgctggagaccagcgagggctgcaggcagatcctgggccagctgcagcccagcctgcagaccggcagcgaggagctgaggagcctgtacaacaccgtggccaccctgtactgcgtgcaccagaggatcgagatcaaggacaccaaggaggccctggacaagatcgaggaggagcagaacaagtccaagaagaaggcccagcaggccgccgccgacaccggccacagcagccaggtgagccagaactaccccatcgtgcagaacatccagggccagatggtgcaccaggccatcagccccaggaccctgaacgcctgggtgaaggtggtggaggagaaggccttcagccccgaggtgatccccatgttcagcgccctgagcgagggagccaccccccaggacctgaacaccatgctgaacaccgtgggcggccaccaggccgccatgcagatgctgaaggagaccatcaacgaggaggccgccgagtgggacagggtgcaccccgtgcacgccggccccatcgcccccggccagatgagggagccccgcggcagcgacatcgccggcaccaccagcaccctgcaggagcagatcggctggatgaccaacaacccccccatccccgtgggcgaaatctacaagaggtggatcatcctgggcctgaacaagatcgtgaggatgtacagccccaccagcatcctggatatcaggcagggccccaaagagcccttcagggactacgtggacaggttctacaagaccctgcgcgccgagcaggccagccaggaggtgaagaactggatgaccgagaccctgctggtgcagaacgccaaccccgactgcaagaccatcctgaaggccctgggacccgccgccaccctggaggagatgatgaccgcctgccagggcgtgggcggccccggccacaaggccagggtgctggccgaggccatgagccaggtgaccaacaccgccaccatcatgatgcagaggggcaacttcaggaaccagaggaagatggtgaagtgcttcaactgcggcaaggagggccacaccgccaggaactgccgcgcccccaggaagaagggctgctggaagtgcggcaaggagggccaccagatgaaggactgcaccgagaggcaggctaattttttagggaagatctggccttcctacaagggaaggccagggaattttcttcagagcagaccagagccaacagccccaccatttcttcagagcagaccagagccaacagccccaccagaagagagcttcaggtctggggtagagacaacaactccccctcagaagcaggagccgatagacaaggaactgtatcctttaacttccctcagatcactctttggcaacgacccctcgtcacaataaagatcggtggccagctgaaggaggccctgctggacaccggcgccgacgacaccgtgctggaggagatgagcctgcccggcaggtggaagcccaagatgatcggcggcatcggcggcttcatcaaggtgaggcagtacgaccagatcctgatcgagatctgcggccacaaggccatcggcaccgtgctggtgggacctacacctgtgaacatcatcggcaggaacctgctgacccagatcggctgcaccctgaacttccccatcagccccatcgagaccgtgcccgtgaagctgaagcccggcatggacggccctaaggtgaagcagtggcccctgaccgaggagaagatcaaggccctggtggagatctgcaccgagatggagaaggagggcaagatcagcaagatcggccccgagaacccctacaacacccccgtgttcgccatcaagaagaaggacagcaccaagtggaggaagctggtggacttcagggagctgaacaagaggacccaggacttctgggaggtgcagctgggcatcccccaccccgccggcctgaagaagaagaagagcgtgaccgtgctggacgtgggcgacgcctacttcagcgtgcccctggacgaggacttcaggaagtataccgccttcaccatccccagcatcaacaacgagacccccggcatccgctaccagtacaacgtgctgccccagggctggaagggcagccccgccatcttccagagcagcatgacaaagatcctggagcccttcaagaagcagaaccccgacatcgtgatctatcagtacatggacgacctgtacgtgggcagcgacctggagatcggccagcacaggaccaagatcgaggagctgaggcagcacctgctgaggtggggcctgaccacccccgacaagaagcaccagaaggagcccccattcctgtggatgggctacgagctgcaccccgacaagtggaccgtgcagcccatcgtgctgcccgagaaggacagctggaccgtgaacgacattcagaagctggtgggcaagctgaactgggccagccagatctaccccggcatcaaggtgaggcagctgtgcaagctgctgaggggcacaaaggctctgaccgaggtgatccccctgaccgaggaggccgagctggagctggccgagaacagggagatcctgaaggagcccgtgcacggcgtgtactacgaccccagcaaggacctgatcgccgagatccagaagcagggccagggccagtggacctaccagatctaccaggagcccttcaagaacctgaagaccggcaagtacgcccgcatgcgcggcgcccacaccaacgacgtgaagcagctgaccgaggccgtgcagaagatcaccaccgagagcatcgtgatctggggcaagactcctaagttcaagctgcccatccagaaggagacctgggagacctggtggaccgagtactggcaggccacctggattcccgagtgggagttcgtgaacacccctcccctggtgaagctgtggtatcagctggagaaggagcccatcgtgggcgccgagaccttctacgtggacggcgccgccaacagggagaccaagctgggcaaggccggctacgtgaccaacaagggccgccagaaggtggtgcccctgaccaacaccaccaaccagaagaccgagctgcaggctatctacctggccctgcaggactcaggcctggaggtgaacatcgtgaccgacagccagtacgccctgggcatcatccaggcccagcccgacaagagcgagagcgagctggtgaaccagatcatcgagcagctgatcaagaaggagaaggtgtacctggcctgggtgcccgcccacaagggcatcggcggcaacgagcaggtggacaagctggtgagcgccggcatcaggaagatcctgttcctggacggcatcgacaaggcccaggacgagcacgagaagtaccacagcaactggagggctatggctagcgacttcaacctgcctcccgtggtggctaaggagatcgtggccagctgcgacaagtgccagctgaagggcgaggccatgcacggccaggtggactgcagccccggcatctggcagctggtttgcacccacctggagggcaaggtgatcctggtggccgtgcacgtggcctccggctacatcgaggccgaggtgatccccgccgagaccggccaggagaccgcctacttcctgctgaagctggccggccgctggcccgtgaagaccatccacaccgacaacggcagcaacttcaccagcgccaccgtgaaggccgcctgctggtgggccggcatcaagcaggagttcggcatcccctacaacccccagtctcagggcgtggtggagagcatgaacaaggagctgaagaagatcatcggccaggtgagggaccaggccgagcacctgaagaccgccgtgcagatggccgtgttcatccacaacttcaagaggaagggcggcatcggcggctacagcgccggcgagaggatcgtggacatcatcgccaccgacatccagaccaaggagctgcagaagcagatcaccaagatccagaacttcagggtgtactacagggacagcaggaaccctctgtggaagggccccgccaagctgctgtggaagggcgagggcgccgtggtgatccaggacaacagcgacatcaaggtggtgcccaggaggaaggccaagatcatcagggactacggcaagcagatggccggcgacgactgcgtggcctccaggcaggacgaggactga

SEQ ID NO: 2 - DNA, 390 bp, Bacteriophage MS2
  misc_feature: codon sequence of MS2 coat protein
atggcctctaattttactcaatttgtgcttgtcgataatggggggacgggagatgtgaccgttgcccctagcaatttcgcaaatggcgttgcagaatggatctctagcaacagcagaagccaagcgtacaaagtaacgtgttccgttcgccaaagctccgcccaaaaacggaagtatacaataaaggttgaggtgccgaaagtagccactcaaacagttggtggggtagaattgcccgtagcggcatggcggtcatatctcaatatggaactcactatcccaatcttcgccacgaatagcgattgtgagctgatagttaaggctatgcaaggtcttctcaaagatggaaaccctattccatctgctatcgccgccaacagcgggatatac

SEQ ID NO: 3 - RNA, 19 nt, Artificial Sequence
  The sequence is synthetized.
  misc_feature: sequence of RNA identified by the MS2 coat protein
acaugaggaucacccaugu